European Patent Specification EP 3 833 775 B1, published June 25, 2025. Title: USE OF LC-MS/MS TO QUANTITATE PROTEIN BIOMARKERS. Applicant: Regeneron Pharmaceuticals, Inc. E, Sook Yen Qiu, Haibo Li, Ning. The sequence listing filed with the application follows.

SEQUENCE LISTING (41 sequences)

SEQ ID NO: 1 - protein, 245 aa, Homo sapiens
MEGPRGWLVLCVLAISLASMVTEDLCRAPDGKKGEAGRPGRRGRPGLKGEQGEPGAPGIRTGIQGLKGDQGEPGPSGNPGKVGYPGPSGPLGARGIPGIKGTKGSPGNIKDQPRPAFSAIRRNPPMGGNVVIFDTVITNQEEPYQNHSGRFVCTVPGYYYFTFQVLSQWEICLSIVSSSRGQVRRSLGFCDTTNKGLFQVVSGGMVLQLQQGDQVWVEKDPKKGHIYQGSEADSVFSGFLIFPSA

SEQ ID NO: 2 - protein, 253 aa, Homo sapiens
MMMKIPWGSIPVLMLLLLLGLIDISQAQLSCTGPPAIPGIPGIPGTPGPDGQPGTPGIKGEKGLPGLAGDHGEFGEKGDPGIPGNPGKVGPKGPMGPKGGPGAPGAPGPKGESGDYKATQKIAFSATRTINVPLRRDQTIRFDHVITNMNNNYEPRSGKFTCKVPGLYYFTYHASSRGNLCVNLMRGRERAQKVVTFCDYAYNTFQVTTGGMVLKLEQGENVFLQATDKNSLLGMEGANSIFSGFLLFPDMEA

SEQ ID NO: 3 - protein, 245 aa, Homo sapiens
MDVGPSSLPHLGLKLLLLLLLLPLRGQANTGCYGIPGMPGLPGAPGKDGYDGLPGPKGEPGIPAIPGIRGPKGQKGEPGLPGHPGKNGPMGPPGMPGVPGPMGIPGEPGEEGRYKQKFQSVFTVTRQTHQPPAPNSLIRFNAVLTNPQGDYDTSTGKFTCKVPGLYYFVYHASHTANLCVLLYRSGVKVVTFCGHTSKTNQVNSGGVLLRLQVGEEVWLAVNDYYDMVGIQGSDSVFSGFLLFPD

SEQ ID NO: 4 - protein, 245 aa, Macaca fascicularis
MEGPQGWLVVCVLAISLASIVTQNVCRAPDGKNGVAGRPGRPGRPGLKGERGEPGAPGIRTGIQGLKGDQGEPGPSGNPGKVGYPGPSGPLGDRGIPGIKGIKGNPGNIKDQPRPAFSAIRRNPPMGGNVVIFDMVITNQEEPYQNHSGRFVCTVPGYYYFTFQVVSEREICLSIVSSSRGQVRRSLGFCDTTNKGLFQVVSGGMVLQLQRGDQVWVEKDPRKGNIYQGLEADSVFSGFLIFPSS

SEQ ID NO: 5 - protein, 253 aa, Macaca fascicularis
MMMKILWGSIPVLMLLLLLGLLDVSWAQGSCTGPPAIPGTPGIPGTPGSDGQPGTPGIKGEKGLPGLAGDHGEFGEKGDPGIPGNPGKVGPKGPMGPKGGPGAPGAPGPKGESGDYKATQKIAFSATRTVNTPLRRDQTIRFDHVITNMNNNYEPRSGKFTCRVPGLYYFTYHASSRGNLCVKLMRGRERPQKVVTFCDYAYNTFQVTTGGMVLKLEQGENVFLQATDKNSLLGMEGANSIFSGFLLFPDVEA

SEQ ID NO: 6 - protein, 245 aa, Macaca fascicularis
MDVGPSSLPHLGLKLLLLLLLLPLRGQANTGCYGIPGMPGLPGAPGKDGHDGLPGPKGEPGIPAIPGTRGPKGQKGEPGTPGHPGKNGPMGPPGMPGVPGPMGIPGEPGEEGRYKQKYQSVFTVARQTHQPPAPNSLIRFNAVLTNPQGDYDTSTGKFTCKVPGLYYFVYHASHTANLCVLLYRGGVKVVTFCGHTSQANQVNSGGVLLRLQVGEEVWLGVNDYYDMVGIQGSDSVFSGFLLFPD

SEQ ID NO: 7 - protein, 245 aa, Macaca mulatta
MEGPQGWLVVCVLAISLASIVTQNVCRAPDGKNGVAGRPGRPGRPGLKGERGEPGAPGIRTGIQGLKGDQGEPGPSGNPGKVGYPGPSGPLGDRGIPGIKGIKGNPGNIKDQPRPAFSAIRRNPPMGGNVVIFDMVITNQEEPYQNHSGRFVCTVPGYYYFTFQVVSEREICLSIVSSSRGQVRRSLGFCDTTNKGLFQVVSGGMVLQLQRGDQVWVEKDPRKGNIYQGLEADSVFSGFLIFPST

SEQ ID NO: 8 - protein, 253 aa, Macaca mulatta
MMMKILWGSIPVLMLLLLLGLLDVSWAQGSCTGPPAIPGTPGIPGTPGSDGQPGTPGIKGEKGLPGLAGDHGEFGEKGDPGIPGNPGKVGPKGPMGPKGGPGAPGAPGPKGESGDYKATQKIAFSATRTINTPLRRDQTIRFDHVITNMNNNYEPRSGKFTCRVPGLYYFTYHASSRGNLCVKLMRGRERPQKVVTFCDYAYNTFQVTTGGMVLKLEQGENVFLQATDKNSLLGMEGANSIFSGFLLFPDVEA

SEQ ID NO: 9 - protein, 245 aa, Macaca mulatta; identical to SEQ ID NO: 6

SEQ ID NO: 10 - protein, 245 aa, Mus musculus
METSQGWLVACVLTMTLVWTVAEDVCRAPNGKDGAPGNPGRPGRPGLKGERGEPGAAGIRTGIRGFKGDPGESGPPGKPGNVGLPGPSGPLGDSGPQGLKGVKGNPGNIRDQPRPAFSAIRQNPMTLGNVVIFDKVLTNQESPYQNHTGRFICAVPGFYYFNFQVISKWDLCLFIKSSSGGQPRDSLSFSNTNNKGLFQVLAGGTVLQLRRGDEVWIEKDPAKGRIYQGTEADSIFSGFLIFPSA

SEQ ID NO: 11 - protein, 253 aa, Mus musculus
MKTQWGEVWTHLLLLLLGFLHVSWAQSSCTGPPGIPGIPGVPGVPGSDGQPGTPGIKGEKGLPGLAGDLGEFGEKGDPGIPGTPGKVGPKGPVGPKGTPGPSGPRGPKGDSGDYGATQKVAFSALRTINSPLRPNQVIRFEKVITNANENYEPRNGKFTCKVPGLYYFTYHASSRGNLCVNLVRGRDRDSMQKVVTFCDYAQNTFQVTTGGVVLKLEQEEVVHLQATDKNSLLGIEGANSIFTGFLLFPDMDA

SEQ ID NO: 12 - protein, 246 aa, Mus musculus
MVVGPSCQPPCGLCLLLLFLLALPLRSQASAGCYGIPGMPGMPGAPGKDGHDGLQGPKGEPGIPAVPGTRGPKGQKGEPGMPGHRGKNGPRGTSGLPGDPGPRGPPGEPGVEGRYKQKHQSVFTVTRQTTQYPEANALVRFNSVVTNPQGHYNPSTGKFTCEVPGLYYFVYYTSHTANLCVHLNLNLARVASFCDHMFNSKQVSSGGVLLRLQRGDEVWLSVNDYNGMVGIEGSNSVFSGFLLFPD

SEQ ID NO: 13 - protein, 245 aa, Rattus norvegicus
METSQGWLVACVLAVTLVWTVAEDVCRAPNGKDGVAGIPGRPGRPGLKGERGEPGAAGIRTGIRGLKGDMGESGPPGKPGNVGFPGPTGPLGNSGPQGLKGVKGNPGNIRDQPRPAFSAIRQNPPTYGNVVVFDKVLTNQENPYQNRTGHFICAVPGFYYFTFQVISKWDLCLSIVSSSRGQPRNSLGFCDTNSKGLFQVLAGGTVLQLQRGDEVWIEKDPAKGRIYQGTEADSIFSGFLIFPSA

SEQ ID NO: 14 - protein, 253 aa, Rattus norvegicus
MKTQWSEILTPLLLLLLGLLHVSWAQSSCTGSPGIPGVPGIPGVPGSDGKPGTPGIKGEKGLPGLAGDHGELGEKGDAGIPGIPGKVGPKGPVGPKGAPGPPGPRGPKGGSGDYKATQKVAFSALRTVNSALRPNQAIRFEKVITNVNDNYEPRSGKFTCKVPGLYYFTYHASSRGNLCVNIVRGRDRDRMQKVLTFCDYAQNTFQVTTGGVVLKLEQEEVVHLQATDKNSLLGVEGANSIFTGFLLFPDMDV

SEQ ID NO: 15 - protein, 245 aa, Rattus norvegicus
MVVGTSCQPQHGLYLLLLLLALPLRSQANAGCYGIPGMPGLPGTPGKDGHDGLQGPKGEPGIPAIPGTQGPKGQKGEPGMPGHRGKNGPMGTSGSPGDPGPRGPPGEPGEEGRYKQKHQSVFTVTRQTAQYPAANGLVKFNSAITNPQGDYNTNTGKFTCKVPGLYYFVHHTSQTANLCVQLLLNNAKVTSFCDHMSNSKQVSSGGVLLRLQRGDEVWLAVNDYNGMVGTEGSDSVFSGFLLFPD

SEQ ID NO: 16 - protein, 245 aa, Canis lupus
MEAPWGWLALCVLATSLASAVTQDVCRALDGRDGAAGTPGRPGRPGLKGEQGEPGAPGMRTGIRGLKGDQGDPGPPGNPGNMGFPGPSGLMGLPGIPGRRGPKGNPGNIRDQPRPAFSAIRRNPPTGGNVVIFDTVITNQEGPYQNHSGRFICAVPGYYYFTFQVVSKWDICLSIVSSGRAQIRRSLGFCDTNSKGIFQVVSGGMALQLQQGDQVWIEKDPIKGRIYQGPEADSIFSGFLIFPSL

SEQ ID NO: 17 - protein, 250 aa, Canis lupus
MKTPRGGILALLLPLLLGLLEVSWAQSCTGHPAIPGIPGIPGAPGTDGTPGTPGTKGEKGLPGLAGDHGEFGEKGDPGIPGTPGKVGPKGPVGPKGSPGPPGARGAKGESGDYKATQKIAFSAMRTINIPLRRDQTIRFDHIVTNENRNYEPRSGKFTCNVPGIYYFAYHASSRGNLCVNVMRGRERMQKVVTFCDYVQNTFQVTTGSVVLKLSQGENVYLQATDKNSLLGMEGANSIFSGFLLFPDAEA

SEQ ID NO: 18 - protein, 245 aa, Canis lupus
MDTGPSSWPHLGLNLLLLLLALPLGGQASTGCYGIPGMPGLPGAPGKDGHDGLPGPKGEPGIPAIPGTRGPKGQKGEPGTPGYPGKNGPMGTPGIPGVPGPVGPPGEPGEEGRYKQKHQSVFTVTRQTAQYPLANNLVKFNTVITNPQGDYDTSTGKFTCKVPGLYYFVYHTSLTSNLCVHLYRSGTRVTTFCDHMSNSKQVSSGGVLLRLQMGEQVWLAVNDYNGMVGTEGSDSVFSGFLLFPD

SEQ ID NO: 19 - protein, 247 aa, Danio rerio
MQPSAFFAFLWAGALFPFSFCQDECVKHGRNGADGPNGRDGLPGPKGEKGEPALQVKLSSIALEELKGDMGVRGPPGEPGLEGLMGAIGPRGPLGPAGPRGSSVGADGAKASEKPAFSVLRNEASQAQYKQPVTFNDKLSDANDDFQIKTGYFTCKVPGVYYFVFHASSEGRLCLRLKSTSAPPVSLSFCDFNSKSVSLVVSGGAVLTLLKGDKVWIEPFAGDGGVGQMPKRLYAVFNGFLIYRNAE

SEQ ID NO: 20 - protein, 242 aa, Danio rerio
MLFALMSAHVVPQLAIMLLLVTSSMSETCAGNKGFPGTPGIPGVPGTDGKDGAKGEKGDPGENEVQMTGPKGDPGKPGLPGRPGVKGPEGPQGPPGPPGPKGQRGVLSGKVAPDQYFVFSYKKSQKLEKILQDKLVVFDVPLITGIDGVLDGEGYFDVTITGMYYISYQISFQQSACLKIQIGAEEKVKFCDSPKLILGTAASVVLKLNKGDKVSVQSTGESTVFSRDTDCTFTGFMLFPIK

SEQ ID NO: 21 - protein, 244 aa, Danio rerio
MFGGHLILVSLLSASLCLCLASADTCPAGAMPGLPGIPGFPGRDGRQGMKGEKGDLGIPIKPGDTVKKGERGAFGLKGPPGKRGPHGDPGIMGPPGPPGEPGEAGLVDVSGSQLQSAFSVSRHTRIPPDANKVIRFSKVITNPQGHFSTDESKFVCKIPGTYYFVLHASSHDKKLCVILVHDDKNLVSFCDHTQRGSQQVSSGGLSLYLKENEKVWLMTNALNGMYATADRADSVFSGFLIHAH

SEQ ID NO: 22 - protein, 13 aa, Macaca fascicularis
VGYPGPSGPLGAR

SEQ ID NO: 23 - protein, 11 aa, Macaca fascicularis
DQPRPAFSAIR

SEQ ID NO: 24 - protein, 28 aa, Macaca fascicularis
NPPMGGNVVIFDTVITNQEEPYQNHSGR

SEQ ID NO: 25 - protein, 30 aa, Macaca fascicularis
FVCTVPGYYYFTFQVLSQWEICLSIVSSSR

SEQ ID NO: 26 - protein, 10 aa, Macaca fascicularis
SLGFCDTTNK

SEQ ID NO: 27 - protein, 26 aa, Macaca fascicularis
GLFVVSGGMVLQLQQGDQVWVEKDPK

SEQ ID NO: 28 - protein, 22 aa, Macaca fascicularis
GHIYQGSEADSVFSGFLIFPSA

SEQ ID NO: 29 - protein, 7 aa, Macaca fascicularis
IAFSATR

SEQ ID NO: 30 - protein, 8 aa, Macaca fascicularis
TINVPLRR

SEQ ID NO: 31 - protein, 15 aa, Macaca fascicularis
FDHVITNMNNNYEPR

SEQ ID NO: 32 - protein, 14 aa, Macaca fascicularis
VPGLYYFTYHASSR

SEQ ID NO: 33 - protein, 9 aa, Macaca fascicularis
GNLCVNLMR

SEQ ID NO: 34 - protein, 14 aa, Macaca fascicularis
LEQGENVFLQATDK

SEQ ID NO: 35 - protein, 9 aa, Macaca fascicularis
FQSVFTVTR

SEQ ID NO: 36 - protein, 13 aa, Macaca fascicularis
QTHQPPAPNSLIR

SEQ ID NO: 37 - protein, 18 aa, Macaca fascicularis
FNAVLTNPQGDYDTSTGK

SEQ ID NO: 38 - protein, 23 aa, Macaca fascicularis
VPGLYYFVYHASHTANLCVLLYR

SEQ ID NO: 39 - protein, 10 aa, Macaca fascicularis
VVTFCGHTSK

SEQ ID NO: 40 - protein, 12 aa, Macaca fascicularis
TNQVNSGGVLLR

SEQ ID NO: 41 - protein, 10 aa, Artificial Sequence
  Modified Peptide
  MOD_RES (5)..(5): Carbamidomethylation
SLGFCDTTNK